European Patent Application EP 4 692 115 A1, published February 11, 2026. Title: ANTIBODY-FUNCTIONAL SUBSTANCE CONJUGATE, ANTIBODY DERIVATIVE, AND COMPOUND, OR SALTS THEREOF. Applicant: AJINOMOTO CO., INC. Application EP EP24784938.3, filed April 3, 2024. The sequence listing filed with the application follows.

SEQUENCE LISTING (13 sequences)

SEQ ID NO: 1 - protein, 17 aa, synthetic construct
RGNCAYHKGQIIWCTYH

SEQ ID NO: 2 - protein, 4 aa, synthetic construct
GGFG

SEQ ID NO: 3 - protein, 4 aa, synthetic construct
DDVD

SEQ ID NO: 4 - protein, 4 aa, synthetic construct
EEVC

SEQ ID NO: 5 - protein, 6 aa, synthetic construct
EEEEVC

SEQ ID NO: 6 - protein, 5 aa, synthetic construct
EGGFG

SEQ ID NO: 7 - protein, 4 aa, synthetic construct
EEFK

SEQ ID NO: 8 - protein, 4 aa, synthetic construct
EEVK

SEQ ID NO: 9 - protein, 4 aa, synthetic construct
EEAK

SEQ ID NO: 10 - protein, 5 aa, synthetic construct
EEVLK

SEQ ID NO: 11 - protein, 5 aa, synthetic construct
EDDVD

SEQ ID NO: 12 - protein, 4 aa, synthetic construct
EEGC

SEQ ID NO: 13 - protein, 34 aa, synthetic construct
FNMQCQRRFYEALHDPNLNEEQRNARIRSIKEEC